European Patent Application EP 4 653 468 A1, published November 26, 2025. Title: DR5 DOMAIN VARIANT AND USE THEREOF. Applicant: SUZHOU YOUTHEN BIOTECHNOLOGY CO.,LTD. The sequence listing filed with the application follows.

SEQUENCE LISTING (99 sequences)

SEQ ID NO: 1 - protein, 127 aa, synthetic construct
  REGION 1..127: note = M3
ITQQDLAPQQRAAPQQKRSSPSEGLCPPGHHISEDGRDCISCKYGQDYSTHWNDLLFCAACTRCDSGEVELSPCTTTRNTVCQCEEGTFREEDSPEMCRKCRTGCPRGMVKVGDCTPWSDIECVHKE

SEQ ID NO: 2 - protein, 127 aa, synthetic construct
  REGION 1..127: note = M5
ITQQDLAPQQRAAPQQKRSSPSEGLCPPGHHISEDGRDCISCKYGQDYSTHWNDLLFCLRCTRCDSGEVELSPCTTTRNTVCQCEEGTFREEDSPEMCAACRTGCPRGMVKVGDCTPWSDIECVHKE

SEQ ID NO: 3 - protein, 127 aa, synthetic construct
  REGION 1..127: note = M14
ITQQDLAPQQRAAPQQKRSSPSEGLCPPGHHLSESGRDCISCKYGQDYSNHWNHLLFCLRCTRCDSGEVELSPCTTTRNTVCQCEEGTFREENSPEMCRKCRTGCPRGMVKVGDCTPWSDIECVHKE

SEQ ID NO: 4 - protein, 127 aa, synthetic construct
  REGION 1..127: note = M16
ITQQDLAPQQRAAPQQKRSSPSEGLCPPGHHASESGRDCISCKYGQDYSNHWNSLLFCVRCTRCDSGEVELSPCTTTRNTVCQCEEGTFRESDSPEMCRKCRTGCPRGMVKVGDCTPWSDIECVHKE

SEQ ID NO: 5 - protein, 127 aa, synthetic construct
  REGION 1..127: note = M29
ITQQDLAPQQRAAPQQKRSSPSEGLCPPGHHASNNGRDCISCKYGQDYSTHWNQLLFCLRCTRCDSGEVELSPCTTTRNTVCQCEEGTFREYDSPEMCRKCRTGCPRGMVKVGDCTPWSDIECVHKE

SEQ ID NO: 6 - protein, 127 aa, synthetic construct
  REGION 1..127: note = M36
ITQQDLAPQQRAAPQQKRSSPSEGLCPPGHHASQSGRDCISCKYGQDYSSHWNSLLFCVRCTRCDSGEVELSPCTTTRNTVCQCEEGTFREEKSPEMCRKCRTGCPRGMVKVGDCTPWSDIECVHKE

SEQ ID NO: 7 - protein, 127 aa, synthetic construct
  REGION 1..127: note = M42
ITQQDLAPQQRAAPQQKRSSPSEGLCPPGHHISESGRDCISCKYGQDYSNHWNELLFCIRCTRCDSGEVELSPCTTTRNTVCQCEEGTFREEESPEMCYKCRTGCPRGMVKVGDCTPWSDIECVHKE

SEQ ID NO: 8 - protein, 127 aa, synthetic construct
  REGION 1..127: note = M47
ITQQDLAPQQRAAPQQKRSSPSEGLCPPGHHISESGRDCISCKYGQDYSTHWNNLLFCLRCTRCDSGEVELSPCTTTRNTVCQCEEGTFREEESPEMCRKCRTGCPRGMVKVGDCTPWSDIECVHKE

SEQ ID NO: 9 - protein, 127 aa, synthetic construct
  REGION 1..127: note = M51
ITQQDLAPQQRAAPQQKRSSPSEGLCPPGHHVSENGRDCISCKYGQDYSTHWNDLLFCLRCTRCDSGEVELSPCTTTRNTVCQCEEGTFREEDSPEMCYKCRTGCPRGMVKVGDCTPWSDIECVHKE

SEQ ID NO: 10 - protein, 127 aa, synthetic construct
  REGION 1..127: note = M52
ITQQDLAPQQRAAPQQKRSSPSEGLCPPGHHISEDGRDCISCKYGQDYSSHWQDLLYCLRCTRCDSGEVELSPCTTTRNTVCQCEEGTFREEDSPEMCRKCRTGCPRGMVKVGDCTPWSDIECVHKE

SEQ ID NO: 11 - protein, 127 aa, synthetic construct
  REGION 1..127: note = M54
ITQQDLAPQQRAAPQQKRSSPSEGLCPPGHHISEDGRDCISCKYGQDYSTHWNDLLFCVRCTRCDSGEVELSPCTTTRNTVCQCEEGTFREQDSPSMCRKCRTGCPRGMVKVGDCTPWSDIECVHKE

SEQ ID NO: 12 - protein, 127 aa, synthetic construct
  REGION 1..127: note = M62
ITQQDLAPQQRAAPQQKRSSPSEGLCPPGHHISEDGRDCISCKYGQDYSTHWNDLLFCGGCTRCDSGEVELSPCTTTRNTVCQCEEGTFREEDSPEMCRKCRTGCPRGMVKVGDCTPWSDIECVHKE

SEQ ID NO: 13 - protein, 127 aa, synthetic construct
  REGION 1..127: note = M63
ITQQDLAPQQRAAPQQKRSSPSEGLCPPGHHISEDGRDCISCKYGQDYSTHWNDLLFCVVCTRCDSGEVELSPCTTTRNTVCQCEEGTFREEDSPEMCRKCRTGCPRGMVKVGDCTPWSDIECVHKE

SEQ ID NO: 14 - protein, 127 aa, synthetic construct
  REGION 1..127: note = M64
ITQQDLAPQQRAAPQQKRSSPSEGLCPPGHHISEDGRDCISCKYGQDYSTHWNDLLFCLLCTRCDSGEVELSPCTTTRNTVCQCEEGTFREEDSPEMCRKCRTGCPRGMVKVGDCTPWSDIECVHKE

SEQ ID NO: 15 - protein, 127 aa, synthetic construct
  REGION 1..127: note = M65
ITQQDLAPQQRAAPQQKRSSPSEGLCPPGHHISEDGRDCISCKYGQDYSTHWNDLLFCSSCTRCDSGEVELSPCTTTRNTVCQCEEGTFREEDSPEMCRKCRTGCPRGMVKVGDCTPWSDIECVHKE

SEQ ID NO: 16 - protein, 127 aa, synthetic construct
  REGION 1..127: note = M66
ITQQDLAPQQRAAPQQKRSSPSEGLCPPGHHISEDGRDCISCKYGQDYSTHWNDLLFCWWCTRCDSGEVELSPCTTTRNTVCQCEEGTFREEDSPEMCRKCRTGCPRGMVKVGDCTPWSDIECVHKE

SEQ ID NO: 17 - protein, 127 aa, synthetic construct
  REGION 1..127: note = M67
ITQQDLAPQQRAAPQQKRSSPSEGLCPPGHHISEDGRDCISCKYGQDYSTHWNDLLFCYYCTRCDSGEVELSPCTTTRNTVCQCEEGTFREEDSPEMCRKCRTGCPRGMVKVGDCTPWSDIECVHKE

SEQ ID NO: 18 - protein, 127 aa, synthetic construct
  REGION 1..127: note = M82
ITQQDLAPQQRAAPQQKRSSPSEGLCPPGHHISEDGRDCISCKYGQDYSTHWNDLLFCLRCTRCDSGEVELSPCTTTRNTVCQCEEGTFREEDSPEMCGGCRTGCPRGMVKVGDCTPWSDIECVHKE

SEQ ID NO: 19 - protein, 127 aa, synthetic construct
  REGION 1..127: note = M83
ITQQDLAPQQRAAPQQKRSSPSEGLCPPGHHISEDGRDCISCKYGQDYSTHWNDLLFCLRCTRCDSGEVELSPCTTTRNTVCQCEEGTFREEDSPEMCVVCRTGCPRGMVKVGDCTPWSDIECVHKE

SEQ ID NO: 20 - protein, 127 aa, synthetic construct
  REGION 1..127: note = M84
ITQQDLAPQQRAAPQQKRSSPSEGLCPPGHHISEDGRDCISCKYGQDYSTHWNDLLFCLRCTRCDSGEVELSPCTTTRNTVCQCEEGTFREEDSPEMCLLCRTGCPRGMVKVGDCTPWSDIECVHKE

SEQ ID NO: 21 - protein, 127 aa, synthetic construct
  REGION 1..127: note = M85
ITQQDLAPQQRAAPQQKRSSPSEGLCPPGHHISEDGRDCISCKYGQDYSTHWNDLLFCLRCTRCDSGEVELSPCTTTRNTVCQCEEGTFREEDSPEMCSSCRTGCPRGMVKVGDCTPWSDIECVHKE

SEQ ID NO: 22 - protein, 127 aa, synthetic construct
  REGION 1..127: note = M86
ITQQDLAPQQRAAPQQKRSSPSEGLCPPGHHISEDGRDCISCKYGQDYSTHWNDLLFCLRCTRCDSGEVELSPCTTTRNTVCQCEEGTFREEDSPEMCWWCRTGCPRGMVKVGDCTPWSDIECVHKE

SEQ ID NO: 23 - protein, 127 aa, synthetic construct
  REGION 1..127: note = M87
ITQQDLAPQQRAAPQQKRSSPSEGLCPPGHHISEDGRDCISCKYGQDYSTHWNDLLFCLRCTRCDSGEVELSPCTTTRNTVCQCEEGTFREEDSPEMCYYCRTGCPRGMVKVGDCTPWSDIECVHKE

SEQ ID NO: 24 - protein, 361 aa, synthetic construct
  REGION 1..361: note = YF01M3
ITQQDLAPQQRAAPQQKRSSPSEGLCPPGHHISEDGRDCISCKYGQDYSTHWNDLLFCAACTRCDSGEVELSPCTTTRNTVCQCEEGTFREEDSPEMCRKCRTGCPRGMVKVGDCTPWSDIECVHKEEFEPKSCDKTHTCPPCPAPELLGGPSVFLFPPKPKDTLMISRTPEVTCVVVDVSHEDPEVKFNWYVDGVEVHNAKTKPREEQYNSTYRVVSVLTVLHQDWLNGKEYKCKVSNKALPAPIEKTISKAKGQPREPQVYTLPPSRDELTKNQVSLTCLVKGFYPSDIAVEWESNGQPENNYKTTPPVLDSDGSFFLYSKLTVDKSRWQQGNVFSCSVMHEALHNHYTQKSLSLSPGK

SEQ ID NO: 25 - protein, 361 aa, synthetic construct
  REGION 1..361: note = YF01M5
ITQQDLAPQQRAAPQQKRSSPSEGLCPPGHHISEDGRDCISCKYGQDYSTHWNDLLFCLRCTRCDSGEVELSPCTTTRNTVCQCEEGTFREEDSPEMCAACRTGCPRGMVKVGDCTPWSDIECVHKEEFEPKSCDKTHTCPPCPAPELLGGPSVFLFPPKPKDTLMISRTPEVTCVVVDVSHEDPEVKFNWYVDGVEVHNAKTKPREEQYNSTYRVVSVLTVLHQDWLNGKEYKCKVSNKALPAPIEKTISKAKGQPREPQVYTLPPSRDELTKNQVSLTCLVKGFYPSDIAVEWESNGQPENNYKTTPPVLDSDGSFFLYSKLTVDKSRWQQGNVFSCSVMHEALHNHYTQKSLSLSPGK

SEQ ID NO: 26 - protein, 361 aa, synthetic construct
  REGION 1..361: note = YF01M14
ITQQDLAPQQRAAPQQKRSSPSEGLCPPGHHLSESGRDCISCKYGQDYSNHWNHLLFCLRCTRCDSGEVELSPCTTTRNTVCQCEEGTFREENSPEMCRKCRTGCPRGMVKVGDCTPWSDIECVHKEEFEPKSCDKTHTCPPCPAPELLGGPSVFLFPPKPKDTLMISRTPEVTCVVVDVSHEDPEVKFNWYVDGVEVHNAKTKPREEQYNSTYRVVSVLTVLHQDWLNGKEYKCKVSNKALPAPIEKTISKAKGQPREPQVYTLPPSRDELTKNQVSLTCLVKGFYPSDIAVEWESNGQPENNYKTTPPVLDSDGSFFLYSKLTVDKSRWQQGNVFSCSVMHEALHNHYTQKSLSLSPGK

SEQ ID NO: 27 - protein, 361 aa, synthetic construct
  REGION 1..361: note = YF01M16
ITQQDLAPQQRAAPQQKRSSPSEGLCPPGHHASESGRDCISCKYGQDYSNHWNSLLFCVRCTRCDSGEVELSPCTTTRNTVCQCEEGTFRESDSPEMCRKCRTGCPRGMVKVGDCTPWSDIECVHKEEFEPKSCDKTHTCPPCPAPELLGGPSVFLFPPKPKDTLMISRTPEVTCVVVDVSHEDPEVKFNWYVDGVEVHNAKTKPREEQYNSTYRVVSVLTVLHQDWLNGKEYKCKVSNKALPAPIEKTISKAKGQPREPQVYTLPPSRDELTKNQVSLTCLVKGFYPSDIAVEWESNGQPENNYKTTPPVLDSDGSFFLYSKLTVDKSRWQQGNVFSCSVMHEALHNHYTQKSLSLSPGK

SEQ ID NO: 28 - protein, 361 aa, synthetic construct
  REGION 1..361: note = YF01M29
ITQQDLAPQQRAAPQQKRSSPSEGLCPPGHHASNNGRDCISCKYGQDYSTHWNQLLFCLRCTRCDSGEVELSPCTTTRNTVCQCEEGTFREYDSPEMCRKCRTGCPRGMVKVGDCTPWSDIECVHKEEFEPKSCDKTHTCPPCPAPELLGGPSVFLFPPKPKDTLMISRTPEVTCVVVDVSHEDPEVKFNWYVDGVEVHNAKTKPREEQYNSTYRVVSVLTVLHQDWLNGKEYKCKVSNKALPAPIEKTISKAKGQPREPQVYTLPPSRDELTKNQVSLTCLVKGFYPSDIAVEWESNGQPENNYKTTPPVLDSDGSFFLYSKLTVDKSRWQQGNVFSCSVMHEALHNHYTQKSLSLSPGK

SEQ ID NO: 29 - protein, 361 aa, synthetic construct
  REGION 1..361: note = YF01M36
ITQQDLAPQQRAAPQQKRSSPSEGLCPPGHHASQSGRDCISCKYGQDYSSHWNSLLFCVRCTRCDSGEVELSPCTTTRNTVCQCEEGTFREEKSPEMCRKCRTGCPRGMVKVGDCTPWSDIECVHKEEFEPKSCDKTHTCPPCPAPELLGGPSVFLFPPKPKDTLMISRTPEVTCVVVDVSHEDPEVKFNWYVDGVEVHNAKTKPREEQYNSTYRVVSVLTVLHQDWLNGKEYKCKVSNKALPAPIEKTISKAKGQPREPQVYTLPPSRDELTKNQVSLTCLVKGFYPSDIAVEWESNGQPENNYKTTPPVLDSDGSFFLYSKLTVDKSRWQQGNVFSCSVMHEALHNHYTQKSLSLSPGK

SEQ ID NO: 30 - protein, 361 aa, synthetic construct
  REGION 1..361: note = YF01M42
ITQQDLAPQQRAAPQQKRSSPSEGLCPPGHHISESGRDCISCKYGQDYSNHWNELLFCIRCTRCDSGEVELSPCTTTRNTVCQCEEGTFREEESPEMCYKCRTGCPRGMVKVGDCTPWSDIECVHKEEFEPKSCDKTHTCPPCPAPELLGGPSVFLFPPKPKDTLMISRTPEVTCVVVDVSHEDPEVKFNWYVDGVEVHNAKTKPREEQYNSTYRVVSVLTVLHQDWLNGKEYKCKVSNKALPAPIEKTISKAKGQPREPQVYTLPPSRDELTKNQVSLTCLVKGFYPSDIAVEWESNGQPENNYKTTPPVLDSDGSFFLYSKLTVDKSRWQQGNVFSCSVMHEALHNHYTQKSLSLSPGK

SEQ ID NO: 31 - protein, 361 aa, synthetic construct
  REGION 1..361: note = YF01M47
ITQQDLAPQQRAAPQQKRSSPSEGLCPPGHHISESGRDCISCKYGQDYSTHWNNLLFCLRCTRCDSGEVELSPCTTTRNTVCQCEEGTFREEESPEMCRKCRTGCPRGMVKVGDCTPWSDIECVHKEEFEPKSCDKTHTCPPCPAPELLGGPSVFLFPPKPKDTLMISRTPEVTCVVVDVSHEDPEVKFNWYVDGVEVHNAKTKPREEQYNSTYRVVSVLTVLHQDWLNGKEYKCKVSNKALPAPIEKTISKAKGQPREPQVYTLPPSRDELTKNQVSLTCLVKGFYPSDIAVEWESNGQPENNYKTTPPVLDSDGSFFLYSKLTVDKSRWQQGNVFSCSVMHEALHNHYTQKSLSLSPGK

SEQ ID NO: 32 - protein, 361 aa, synthetic construct
  REGION 1..361: note = YF01M51
ITQQDLAPQQRAAPQQKRSSPSEGLCPPGHHVSENGRDCISCKYGQDYSTHWNDLLFCLRCTRCDSGEVELSPCTTTRNTVCQCEEGTFREEDSPEMCYKCRTGCPRGMVKVGDCTPWSDIECVHKEEFEPKSCDKTHTCPPCPAPELLGGPSVFLFPPKPKDTLMISRTPEVTCVVVDVSHEDPEVKFNWYVDGVEVHNAKTKPREEQYNSTYRVVSVLTVLHQDWLNGKEYKCKVSNKALPAPIEKTISKAKGQPREPQVYTLPPSRDELTKNQVSLTCLVKGFYPSDIAVEWESNGQPENNYKTTPPVLDSDGSFFLYSKLTVDKSRWQQGNVFSCSVMHEALHNHYTQKSLSLSPGK

SEQ ID NO: 33 - protein, 361 aa, synthetic construct
  REGION 1..361: note = YF01M52
ITQQDLAPQQRAAPQQKRSSPSEGLCPPGHHISEDGRDCISCKYGQDYSSHWQDLLYCLRCTRCDSGEVELSPCTTTRNTVCQCEEGTFREEDSPEMCRKCRTGCPRGMVKVGDCTPWSDIECVHKEEFEPKSCDKTHTCPPCPAPELLGGPSVFLFPPKPKDTLMISRTPEVTCVVVDVSHEDPEVKFNWYVDGVEVHNAKTKPREEQYNSTYRVVSVLTVLHQDWLNGKEYKCKVSNKALPAPIEKTISKAKGQPREPQVYTLPPSRDELTKNQVSLTCLVKGFYPSDIAVEWESNGQPENNYKTTPPVLDSDGSFFLYSKLTVDKSRWQQGNVFSCSVMHEALHNHYTQKSLSLSPGK

SEQ ID NO: 34 - protein, 361 aa, synthetic construct
  REGION 1..361: note = YF01M54
ITQQDLAPQQRAAPQQKRSSPSEGLCPPGHHISEDGRDCISCKYGQDYSTHWNDLLFCVRCTRCDSGEVELSPCTTTRNTVCQCEEGTFREQDSPSMCRKCRTGCPRGMVKVGDCTPWSDIECVHKEEFEPKSCDKTHTCPPCPAPELLGGPSVFLFPPKPKDTLMISRTPEVTCVVVDVSHEDPEVKFNWYVDGVEVHNAKTKPREEQYNSTYRVVSVLTVLHQDWLNGKEYKCKVSNKALPAPIEKTISKAKGQPREPQVYTLPPSRDELTKNQVSLTCLVKGFYPSDIAVEWESNGQPENNYKTTPPVLDSDGSFFLYSKLTVDKSRWQQGNVFSCSVMHEALHNHYTQKSLSLSPGK

SEQ ID NO: 35 - protein, 361 aa, synthetic construct
  REGION 1..361: note = YF01M62
ITQQDLAPQQRAAPQQKRSSPSEGLCPPGHHISEDGRDCISCKYGQDYSTHWNDLLFCGGCTRCDSGEVELSPCTTTRNTVCQCEEGTFREEDSPEMCRKCRTGCPRGMVKVGDCTPWSDIECVHKEEFEPKSCDKTHTCPPCPAPELLGGPSVFLFPPKPKDTLMISRTPEVTCVVVDVSHEDPEVKFNWYVDGVEVHNAKTKPREEQYNSTYRVVSVLTVLHQDWLNGKEYKCKVSNKALPAPIEKTISKAKGQPREPQVYTLPPSRDELTKNQVSLTCLVKGFYPSDIAVEWESNGQPENNYKTTPPVLDSDGSFFLYSKLTVDKSRWQQGNVFSCSVMHEALHNHYTQKSLSLSPGK

SEQ ID NO: 36 - protein, 361 aa, synthetic construct
  REGION 1..361: note = YF01M63
ITQQDLAPQQRAAPQQKRSSPSEGLCPPGHHISEDGRDCISCKYGQDYSTHWNDLLFCVVCTRCDSGEVELSPCTTTRNTVCQCEEGTFREEDSPEMCRKCRTGCPRGMVKVGDCTPWSDIECVHKEEFEPKSCDKTHTCPPCPAPELLGGPSVFLFPPKPKDTLMISRTPEVTCVVVDVSHEDPEVKFNWYVDGVEVHNAKTKPREEQYNSTYRVVSVLTVLHQDWLNGKEYKCKVSNKALPAPIEKTISKAKGQPREPQVYTLPPSRDELTKNQVSLTCLVKGFYPSDIAVEWESNGQPENNYKTTPPVLDSDGSFFLYSKLTVDKSRWQQGNVFSCSVMHEALHNHYTQKSLSLSPGK

SEQ ID NO: 37 - protein, 361 aa, synthetic construct
  REGION 1..361: note = YF01M64
ITQQDLAPQQRAAPQQKRSSPSEGLCPPGHHISEDGRDCISCKYGQDYSTHWNDLLFCLLCTRCDSGEVELSPCTTTRNTVCQCEEGTFREEDSPEMCRKCRTGCPRGMVKVGDCTPWSDIECVHKEEFEPKSCDKTHTCPPCPAPELLGGPSVFLFPPKPKDTLMISRTPEVTCVVVDVSHEDPEVKFNWYVDGVEVHNAKTKPREEQYNSTYRVVSVLTVLHQDWLNGKEYKCKVSNKALPAPIEKTISKAKGQPREPQVYTLPPSRDELTKNQVSLTCLVKGFYPSDIAVEWESNGQPENNYKTTPPVLDSDGSFFLYSKLTVDKSRWQQGNVFSCSVMHEALHNHYTQKSLSLSPGK

SEQ ID NO: 38 - protein, 361 aa, synthetic construct
  REGION 1..361: note = YF01M65
ITQQDLAPQQRAAPQQKRSSPSEGLCPPGHHISEDGRDCISCKYGQDYSTHWNDLLFCSSCTRCDSGEVELSPCTTTRNTVCQCEEGTFREEDSPEMCRKCRTGCPRGMVKVGDCTPWSDIECVHKEEFEPKSCDKTHTCPPCPAPELLGGPSVFLFPPKPKDTLMISRTPEVTCVVVDVSHEDPEVKFNWYVDGVEVHNAKTKPREEQYNSTYRVVSVLTVLHQDWLNGKEYKCKVSNKALPAPIEKTISKAKGQPREPQVYTLPPSRDELTKNQVSLTCLVKGFYPSDIAVEWESNGQPENNYKTTPPVLDSDGSFFLYSKLTVDKSRWQQGNVFSCSVMHEALHNHYTQKSLSLSPGK

SEQ ID NO: 39 - protein, 361 aa, synthetic construct
  REGION 1..361: note = YF01M66
ITQQDLAPQQRAAPQQKRSSPSEGLCPPGHHISEDGRDCISCKYGQDYSTHWNDLLFCWWCTRCDSGEVELSPCTTTRNTVCQCEEGTFREEDSPEMCRKCRTGCPRGMVKVGDCTPWSDIECVHKEEFEPKSCDKTHTCPPCPAPELLGGPSVFLFPPKPKDTLMISRTPEVTCVVVDVSHEDPEVKFNWYVDGVEVHNAKTKPREEQYNSTYRVVSVLTVLHQDWLNGKEYKCKVSNKALPAPIEKTISKAKGQPREPQVYTLPPSRDELTKNQVSLTCLVKGFYPSDIAVEWESNGQPENNYKTTPPVLDSDGSFFLYSKLTVDKSRWQQGNVFSCSVMHEALHNHYTQKSLSLSPGK

SEQ ID NO: 40 - protein, 361 aa, synthetic construct
  REGION 1..361: note = YF01M67
ITQQDLAPQQRAAPQQKRSSPSEGLCPPGHHISEDGRDCISCKYGQDYSTHWNDLLFCYYCTRCDSGEVELSPCTTTRNTVCQCEEGTFREEDSPEMCRKCRTGCPRGMVKVGDCTPWSDIECVHKEEFEPKSCDKTHTCPPCPAPELLGGPSVFLFPPKPKDTLMISRTPEVTCVVVDVSHEDPEVKFNWYVDGVEVHNAKTKPREEQYNSTYRVVSVLTVLHQDWLNGKEYKCKVSNKALPAPIEKTISKAKGQPREPQVYTLPPSRDELTKNQVSLTCLVKGFYPSDIAVEWESNGQPENNYKTTPPVLDSDGSFFLYSKLTVDKSRWQQGNVFSCSVMHEALHNHYTQKSLSLSPGK

SEQ ID NO: 41 - protein, 361 aa, synthetic construct
  REGION 1..361: note = YF01M82
ITQQDLAPQQRAAPQQKRSSPSEGLCPPGHHISEDGRDCISCKYGQDYSTHWNDLLFCLRCTRCDSGEVELSPCTTTRNTVCQCEEGTFREEDSPEMCGGCRTGCPRGMVKVGDCTPWSDIECVHKEEFEPKSCDKTHTCPPCPAPELLGGPSVFLFPPKPKDTLMISRTPEVTCVVVDVSHEDPEVKFNWYVDGVEVHNAKTKPREEQYNSTYRVVSVLTVLHQDWLNGKEYKCKVSNKALPAPIEKTISKAKGQPREPQVYTLPPSRDELTKNQVSLTCLVKGFYPSDIAVEWESNGQPENNYKTTPPVLDSDGSFFLYSKLTVDKSRWQQGNVFSCSVMHEALHNHYTQKSLSLSPGK

SEQ ID NO: 42 - protein, 361 aa, synthetic construct
  REGION 1..361: note = YF01M83
ITQQDLAPQQRAAPQQKRSSPSEGLCPPGHHISEDGRDCISCKYGQDYSTHWNDLLFCLRCTRCDSGEVELSPCTTTRNTVCQCEEGTFREEDSPEMCVVCRTGCPRGMVKVGDCTPWSDIECVHKEEFEPKSCDKTHTCPPCPAPELLGGPSVFLFPPKPKDTLMISRTPEVTCVVVDVSHEDPEVKFNWYVDGVEVHNAKTKPREEQYNSTYRVVSVLTVLHQDWLNGKEYKCKVSNKALPAPIEKTISKAKGQPREPQVYTLPPSRDELTKNQVSLTCLVKGFYPSDIAVEWESNGQPENNYKTTPPVLDSDGSFFLYSKLTVDKSRWQQGNVFSCSVMHEALHNHYTQKSLSLSPGK

SEQ ID NO: 43 - protein, 361 aa, synthetic construct
  REGION 1..361: note = YF01M84
ITQQDLAPQQRAAPQQKRSSPSEGLCPPGHHISEDGRDCISCKYGQDYSTHWNDLLFCLRCTRCDSGEVELSPCTTTRNTVCQCEEGTFREEDSPEMCLLCRTGCPRGMVKVGDCTPWSDIECVHKEEFEPKSCDKTHTCPPCPAPELLGGPSVFLFPPKPKDTLMISRTPEVTCVVVDVSHEDPEVKFNWYVDGVEVHNAKTKPREEQYNSTYRVVSVLTVLHQDWLNGKEYKCKVSNKALPAPIEKTISKAKGQPREPQVYTLPPSRDELTKNQVSLTCLVKGFYPSDIAVEWESNGQPENNYKTTPPVLDSDGSFFLYSKLTVDKSRWQQGNVFSCSVMHEALHNHYTQKSLSLSPGK

SEQ ID NO: 44 - protein, 361 aa, synthetic construct
  REGION 1..361: note = YF01M85
ITQQDLAPQQRAAPQQKRSSPSEGLCPPGHHISEDGRDCISCKYGQDYSTHWNDLLFCLRCTRCDSGEVELSPCTTTRNTVCQCEEGTFREEDSPEMCSSCRTGCPRGMVKVGDCTPWSDIECVHKEEFEPKSCDKTHTCPPCPAPELLGGPSVFLFPPKPKDTLMISRTPEVTCVVVDVSHEDPEVKFNWYVDGVEVHNAKTKPREEQYNSTYRVVSVLTVLHQDWLNGKEYKCKVSNKALPAPIEKTISKAKGQPREPQVYTLPPSRDELTKNQVSLTCLVKGFYPSDIAVEWESNGQPENNYKTTPPVLDSDGSFFLYSKLTVDKSRWQQGNVFSCSVMHEALHNHYTQKSLSLSPGK

SEQ ID NO: 45 - protein, 361 aa, synthetic construct
  REGION 1..361: note = YF01M86
ITQQDLAPQQRAAPQQKRSSPSEGLCPPGHHISEDGRDCISCKYGQDYSTHWNDLLFCLRCTRCDSGEVELSPCTTTRNTVCQCEEGTFREEDSPEMCWWCRTGCPRGMVKVGDCTPWSDIECVHKEEFEPKSCDKTHTCPPCPAPELLGGPSVFLFPPKPKDTLMISRTPEVTCVVVDVSHEDPEVKFNWYVDGVEVHNAKTKPREEQYNSTYRVVSVLTVLHQDWLNGKEYKCKVSNKALPAPIEKTISKAKGQPREPQVYTLPPSRDELTKNQVSLTCLVKGFYPSDIAVEWESNGQPENNYKTTPPVLDSDGSFFLYSKLTVDKSRWQQGNVFSCSVMHEALHNHYTQKSLSLSPGK

SEQ ID NO: 46 - protein, 361 aa, synthetic construct
  REGION 1..361: note = YF01M87
ITQQDLAPQQRAAPQQKRSSPSEGLCPPGHHISEDGRDCISCKYGQDYSTHWNDLLFCLRCTRCDSGEVELSPCTTTRNTVCQCEEGTFREEDSPEMCYYCRTGCPRGMVKVGDCTPWSDIECVHKEEFEPKSCDKTHTCPPCPAPELLGGPSVFLFPPKPKDTLMISRTPEVTCVVVDVSHEDPEVKFNWYVDGVEVHNAKTKPREEQYNSTYRVVSVLTVLHQDWLNGKEYKCKVSNKALPAPIEKTISKAKGQPREPQVYTLPPSRDELTKNQVSLTCLVKGFYPSDIAVEWESNGQPENNYKTTPPVLDSDGSFFLYSKLTVDKSRWQQGNVFSCSVMHEALHNHYTQKSLSLSPGK

SEQ ID NO: 47 - protein, 358 aa, synthetic construct
  REGION 1..358: note = YF01M3G4
ITQQDLAPQQRAAPQQKRSSPSEGLCPPGHHISEDGRDCISCKYGQDYSTHWNDLLFCAACTRCDSGEVELSPCTTTRNTVCQCEEGTFREEDSPEMCRKCRTGCPRGMVKVGDCTPWSDIECVHKEEFESKYGPPCPPCPAPEFLGGPSVFLFPPKPKDTLMISRTPEVTCVVVDVSQEDPEVQFNWYVDGVEVHNAKTKPREEQFNSTYRVVSVLTVLHQDWLNGKEYKCKVSNKGLPSSIEKTISKAKGQPREPQVYTLPPSQEEMTKNQVSLTCLVKGFYPSDIAVEWESNGQPENNYKTTPPVLDSDGSFFLYSRLTVDKSRWQEGNVFSCSVMHEALHNHYTQKSLSLSLGK

SEQ ID NO: 48 - protein, 358 aa, synthetic construct
  REGION 1..358: note = YF01M5G4
ITQQDLAPQQRAAPQQKRSSPSEGLCPPGHHISEDGRDCISCKYGQDYSTHWNDLLFCLRCTRCDSGEVELSPCTTTRNTVCQCEEGTFREEDSPEMCAACRTGCPRGMVKVGDCTPWSDIECVHKEEFESKYGPPCPPCPAPEFLGGPSVFLFPPKPKDTLMISRTPEVTCVVVDVSQEDPEVQFNWYVDGVEVHNAKTKPREEQFNSTYRVVSVLTVLHQDWLNGKEYKCKVSNKGLPSSIEKTISKAKGQPREPQVYTLPPSQEEMTKNQVSLTCLVKGFYPSDIAVEWESNGQPENNYKTTPPVLDSDGSFFLYSRLTVDKSRWQEGNVFSCSVMHEALHNHYTQKSLSLSLGK

SEQ ID NO: 49 - protein, 358 aa, synthetic construct
  REGION 1..358: note = YF01M14G4
ITQQDLAPQQRAAPQQKRSSPSEGLCPPGHHLSESGRDCISCKYGQDYSNHWNHLLFCLRCTRCDSGEVELSPCTTTRNTVCQCEEGTFREENSPEMCRKCRTGCPRGMVKVGDCTPWSDIECVHKEEFESKYGPPCPPCPAPEFLGGPSVFLFPPKPKDTLMISRTPEVTCVVVDVSQEDPEVQFNWYVDGVEVHNAKTKPREEQFNSTYRVVSVLTVLHQDWLNGKEYKCKVSNKGLPSSIEKTISKAKGQPREPQVYTLPPSQEEMTKNQVSLTCLVKGFYPSDIAVEWESNGQPENNYKTTPPVLDSDGSFFLYSRLTVDKSRWQEGNVFSCSVMHEALHNHYTQKSLSLSLGK

SEQ ID NO: 50 - protein, 358 aa, synthetic construct
  REGION 1..358: note = YF01M16G4
ITQQDLAPQQRAAPQQKRSSPSEGLCPPGHHASESGRDCISCKYGQDYSNHWNSLLFCVRCTRCDSGEVELSPCTTTRNTVCQCEEGTFRESDSPEMCRKCRTGCPRGMVKVGDCTPWSDIECVHKEEFESKYGPPCPPCPAPEFLGGPSVFLFPPKPKDTLMISRTPEVTCVVVDVSQEDPEVQFNWYVDGVEVHNAKTKPREEQFNSTYRVVSVLTVLHQDWLNGKEYKCKVSNKGLPSSIEKTISKAKGQPREPQVYTLPPSQEEMTKNQVSLTCLVKGFYPSDIAVEWESNGQPENNYKTTPPVLDSDGSFFLYSRLTVDKSRWQEGNVFSCSVMHEALHNHYTQKSLSLSLGK

SEQ ID NO: 51 - protein, 358 aa, synthetic construct
  REGION 1..358: note = YF01M29G4
ITQQDLAPQQRAAPQQKRSSPSEGLCPPGHHASNNGRDCISCKYGQDYSTHWNQLLFCLRCTRCDSGEVELSPCTTTRNTVCQCEEGTFREYDSPEMCRKCRTGCPRGMVKVGDCTPWSDIECVHKEEFESKYGPPCPPCPAPEFLGGPSVFLFPPKPKDTLMISRTPEVTCVVVDVSQEDPEVQFNWYVDGVEVHNAKTKPREEQFNSTYRVVSVLTVLHQDWLNGKEYKCKVSNKGLPSSIEKTISKAKGQPREPQVYTLPPSQEEMTKNQVSLTCLVKGFYPSDIAVEWESNGQPENNYKTTPPVLDSDGSFFLYSRLTVDKSRWQEGNVFSCSVMHEALHNHYTQKSLSLSLGK

SEQ ID NO: 52 - protein, 358 aa, synthetic construct
  REGION 1..358: note = YF01M36G4
ITQQDLAPQQRAAPQQKRSSPSEGLCPPGHHASQSGRDCISCKYGQDYSSHWNSLLFCVRCTRCDSGEVELSPCTTTRNTVCQCEEGTFREEKSPEMCRKCRTGCPRGMVKVGDCTPWSDIECVHKEEFESKYGPPCPPCPAPEFLGGPSVFLFPPKPKDTLMISRTPEVTCVVVDVSQEDPEVQFNWYVDGVEVHNAKTKPREEQFNSTYRVVSVLTVLHQDWLNGKEYKCKVSNKGLPSSIEKTISKAKGQPREPQVYTLPPSQEEMTKNQVSLTCLVKGFYPSDIAVEWESNGQPENNYKTTPPVLDSDGSFFLYSRLTVDKSRWQEGNVFSCSVMHEALHNHYTQKSLSLSLGK

SEQ ID NO: 53 - protein, 358 aa, synthetic construct
  REGION 1..358: note = YF01M42G4
ITQQDLAPQQRAAPQQKRSSPSEGLCPPGHHISESGRDCISCKYGQDYSNHWNELLFCIRCTRCDSGEVELSPCTTTRNTVCQCEEGTFREEESPEMCYKCRTGCPRGMVKVGDCTPWSDIECVHKEEFESKYGPPCPPCPAPEFLGGPSVFLFPPKPKDTLMISRTPEVTCVVVDVSQEDPEVQFNWYVDGVEVHNAKTKPREEQFNSTYRVVSVLTVLHQDWLNGKEYKCKVSNKGLPSSIEKTISKAKGQPREPQVYTLPPSQEEMTKNQVSLTCLVKGFYPSDIAVEWESNGQPENNYKTTPPVLDSDGSFFLYSRLTVDKSRWQEGNVFSCSVMHEALHNHYTQKSLSLSLGK

SEQ ID NO: 54 - protein, 358 aa, synthetic construct
  REGION 1..358: note = YF01M47G4
ITQQDLAPQQRAAPQQKRSSPSEGLCPPGHHISESGRDCISCKYGQDYSTHWNNLLFCLRCTRCDSGEVELSPCTTTRNTVCQCEEGTFREEESPEMCRKCRTGCPRGMVKVGDCTPWSDIECVHKEEFESKYGPPCPPCPAPEFLGGPSVFLFPPKPKDTLMISRTPEVTCVVVDVSQEDPEVQFNWYVDGVEVHNAKTKPREEQFNSTYRVVSVLTVLHQDWLNGKEYKCKVSNKGLPSSIEKTISKAKGQPREPQVYTLPPSQEEMTKNQVSLTCLVKGFYPSDIAVEWESNGQPENNYKTTPPVLDSDGSFFLYSRLTVDKSRWQEGNVFSCSVMHEALHNHYTQKSLSLSLGK

SEQ ID NO: 55 - protein, 358 aa, synthetic construct
  REGION 1..358: note = YF01M51G4
ITQQDLAPQQRAAPQQKRSSPSEGLCPPGHHVSENGRDCISCKYGQDYSTHWNDLLFCLRCTRCDSGEVELSPCTTTRNTVCQCEEGTFREEDSPEMCYKCRTGCPRGMVKVGDCTPWSDIECVHKEEFESKYGPPCPPCPAPEFLGGPSVFLFPPKPKDTLMISRTPEVTCVVVDVSQEDPEVQFNWYVDGVEVHNAKTKPREEQFNSTYRVVSVLTVLHQDWLNGKEYKCKVSNKGLPSSIEKTISKAKGQPREPQVYTLPPSQEEMTKNQVSLTCLVKGFYPSDIAVEWESNGQPENNYKTTPPVLDSDGSFFLYSRLTVDKSRWQEGNVFSCSVMHEALHNHYTQKSLSLSLGK

SEQ ID NO: 56 - protein, 358 aa, synthetic construct
  REGION 1..358: note = YF01M52G4
ITQQDLAPQQRAAPQQKRSSPSEGLCPPGHHISEDGRDCISCKYGQDYSSHWQDLLYCLRCTRCDSGEVELSPCTTTRNTVCQCEEGTFREEDSPEMCRKCRTGCPRGMVKVGDCTPWSDIECVHKEEFESKYGPPCPPCPAPEFLGGPSVFLFPPKPKDTLMISRTPEVTCVVVDVSQEDPEVQFNWYVDGVEVHNAKTKPREEQFNSTYRVVSVLTVLHQDWLNGKEYKCKVSNKGLPSSIEKTISKAKGQPREPQVYTLPPSQEEMTKNQVSLTCLVKGFYPSDIAVEWESNGQPENNYKTTPPVLDSDGSFFLYSRLTVDKSRWQEGNVFSCSVMHEALHNHYTQKSLSLSLGK

SEQ ID NO: 57 - protein, 358 aa, synthetic construct
  REGION 1..358: note = YF01M54G4
ITQQDLAPQQRAAPQQKRSSPSEGLCPPGHHISEDGRDCISCKYGQDYSTHWNDLLFCVRCTRCDSGEVELSPCTTTRNTVCQCEEGTFREQDSPSMCRKCRTGCPRGMVKVGDCTPWSDIECVHKEEFESKYGPPCPPCPAPEFLGGPSVFLFPPKPKDTLMISRTPEVTCVVVDVSQEDPEVQFNWYVDGVEVHNAKTKPREEQFNSTYRVVSVLTVLHQDWLNGKEYKCKVSNKGLPSSIEKTISKAKGQPREPQVYTLPPSQEEMTKNQVSLTCLVKGFYPSDIAVEWESNGQPENNYKTTPPVLDSDGSFFLYSRLTVDKSRWQEGNVFSCSVMHEALHNHYTQKSLSLSLGK

SEQ ID NO: 58 - protein, 358 aa, synthetic construct
  REGION 1..358: note = YF01M62G4
ITQQDLAPQQRAAPQQKRSSPSEGLCPPGHHISEDGRDCISCKYGQDYSTHWNDLLFCGGCTRCDSGEVELSPCTTTRNTVCQCEEGTFREEDSPEMCRKCRTGCPRGMVKVGDCTPWSDIECVHKEEFESKYGPPCPPCPAPEFLGGPSVFLFPPKPKDTLMISRTPEVTCVVVDVSQEDPEVQFNWYVDGVEVHNAKTKPREEQFNSTYRVVSVLTVLHQDWLNGKEYKCKVSNKGLPSSIEKTISKAKGQPREPQVYTLPPSQEEMTKNQVSLTCLVKGFYPSDIAVEWESNGQPENNYKTTPPVLDSDGSFFLYSRLTVDKSRWQEGNVFSCSVMHEALHNHYTQKSLSLSLGK

SEQ ID NO: 59 - protein, 358 aa, synthetic construct
  REGION 1..358: note = YF01M63G4
ITQQDLAPQQRAAPQQKRSSPSEGLCPPGHHISEDGRDCISCKYGQDYSTHWNDLLFCVVCTRCDSGEVELSPCTTTRNTVCQCEEGTFREEDSPEMCRKCRTGCPRGMVKVGDCTPWSDIECVHKEEFESKYGPPCPPCPAPEFLGGPSVFLFPPKPKDTLMISRTPEVTCVVVDVSQEDPEVQFNWYVDGVEVHNAKTKPREEQFNSTYRVVSVLTVLHQDWLNGKEYKCKVSNKGLPSSIEKTISKAKGQPREPQVYTLPPSQEEMTKNQVSLTCLVKGFYPSDIAVEWESNGQPENNYKTTPPVLDSDGSFFLYSRLTVDKSRWQEGNVFSCSVMHEALHNHYTQKSLSLSLGK

SEQ ID NO: 60 - protein, 358 aa, synthetic construct
  REGION 1..358: note = YF01M64G4
ITQQDLAPQQRAAPQQKRSSPSEGLCPPGHHISEDGRDCISCKYGQDYSTHWNDLLFCLLCTRCDSGEVELSPCTTTRNTVCQCEEGTFREEDSPEMCRKCRTGCPRGMVKVGDCTPWSDIECVHKEEFESKYGPPCPPCPAPEFLGGPSVFLFPPKPKDTLMISRTPEVTCVVVDVSQEDPEVQFNWYVDGVEVHNAKTKPREEQFNSTYRVVSVLTVLHQDWLNGKEYKCKVSNKGLPSSIEKTISKAKGQPREPQVYTLPPSQEEMTKNQVSLTCLVKGFYPSDIAVEWESNGQPENNYKTTPPVLDSDGSFFLYSRLTVDKSRWQEGNVFSCSVMHEALHNHYTQKSLSLSLGK

SEQ ID NO: 61 - protein, 358 aa, synthetic construct
  REGION 1..358: note = YF01M65G4
ITQQDLAPQQRAAPQQKRSSPSEGLCPPGHHISEDGRDCISCKYGQDYSTHWNDLLFCSSCTRCDSGEVELSPCTTTRNTVCQCEEGTFREEDSPEMCRKCRTGCPRGMVKVGDCTPWSDIECVHKEEFESKYGPPCPPCPAPEFLGGPSVFLFPPKPKDTLMISRTPEVTCVVVDVSQEDPEVQFNWYVDGVEVHNAKTKPREEQFNSTYRVVSVLTVLHQDWLNGKEYKCKVSNKGLPSSIEKTISKAKGQPREPQVYTLPPSQEEMTKNQVSLTCLVKGFYPSDIAVEWESNGQPENNYKTTPPVLDSDGSFFLYSRLTVDKSRWQEGNVFSCSVMHEALHNHYTQKSLSLSLGK

SEQ ID NO: 62 - protein, 358 aa, synthetic construct
  REGION 1..358: note = YF01M66G4
ITQQDLAPQQRAAPQQKRSSPSEGLCPPGHHISEDGRDCISCKYGQDYSTHWNDLLFCWWCTRCDSGEVELSPCTTTRNTVCQCEEGTFREEDSPEMCRKCRTGCPRGMVKVGDCTPWSDIECVHKEEFESKYGPPCPPCPAPEFLGGPSVFLFPPKPKDTLMISRTPEVTCVVVDVSQEDPEVQFNWYVDGVEVHNAKTKPREEQFNSTYRVVSVLTVLHQDWLNGKEYKCKVSNKGLPSSIEKTISKAKGQPREPQVYTLPPSQEEMTKNQVSLTCLVKGFYPSDIAVEWESNGQPENNYKTTPPVLDSDGSFFLYSRLTVDKSRWQEGNVFSCSVMHEALHNHYTQKSLSLSLGK

SEQ ID NO: 63 - protein, 358 aa, synthetic construct
  REGION 1..358: note = YF01M67G4
ITQQDLAPQQRAAPQQKRSSPSEGLCPPGHHISEDGRDCISCKYGQDYSTHWNDLLFCYYCTRCDSGEVELSPCTTTRNTVCQCEEGTFREEDSPEMCRKCRTGCPRGMVKVGDCTPWSDIECVHKEEFESKYGPPCPPCPAPEFLGGPSVFLFPPKPKDTLMISRTPEVTCVVVDVSQEDPEVQFNWYVDGVEVHNAKTKPREEQFNSTYRVVSVLTVLHQDWLNGKEYKCKVSNKGLPSSIEKTISKAKGQPREPQVYTLPPSQEEMTKNQVSLTCLVKGFYPSDIAVEWESNGQPENNYKTTPPVLDSDGSFFLYSRLTVDKSRWQEGNVFSCSVMHEALHNHYTQKSLSLSLGK

SEQ ID NO: 64 - protein, 358 aa, synthetic construct
  REGION 1..358: note = YF01M82G4
ITQQDLAPQQRAAPQQKRSSPSEGLCPPGHHISEDGRDCISCKYGQDYSTHWNDLLFCLRCTRCDSGEVELSPCTTTRNTVCQCEEGTFREEDSPEMCGGCRTGCPRGMVKVGDCTPWSDIECVHKEEFESKYGPPCPPCPAPEFLGGPSVFLFPPKPKDTLMISRTPEVTCVVVDVSQEDPEVQFNWYVDGVEVHNAKTKPREEQFNSTYRVVSVLTVLHQDWLNGKEYKCKVSNKGLPSSIEKTISKAKGQPREPQVYTLPPSQEEMTKNQVSLTCLVKGFYPSDIAVEWESNGQPENNYKTTPPVLDSDGSFFLYSRLTVDKSRWQEGNVFSCSVMHEALHNHYTQKSLSLSLGK

SEQ ID NO: 65 - protein, 358 aa, synthetic construct
  REGION 1..358: note = YF01M83G4
ITQQDLAPQQRAAPQQKRSSPSEGLCPPGHHISEDGRDCISCKYGQDYSTHWNDLLFCLRCTRCDSGEVELSPCTTTRNTVCQCEEGTFREEDSPEMCVVCRTGCPRGMVKVGDCTPWSDIECVHKEEFESKYGPPCPPCPAPEFLGGPSVFLFPPKPKDTLMISRTPEVTCVVVDVSQEDPEVQFNWYVDGVEVHNAKTKPREEQFNSTYRVVSVLTVLHQDWLNGKEYKCKVSNKGLPSSIEKTISKAKGQPREPQVYTLPPSQEEMTKNQVSLTCLVKGFYPSDIAVEWESNGQPENNYKTTPPVLDSDGSFFLYSRLTVDKSRWQEGNVFSCSVMHEALHNHYTQKSLSLSLGK

SEQ ID NO: 66 - protein, 358 aa, synthetic construct
  REGION 1..358: note = YF01M84G4
ITQQDLAPQQRAAPQQKRSSPSEGLCPPGHHISEDGRDCISCKYGQDYSTHWNDLLFCLRCTRCDSGEVELSPCTTTRNTVCQCEEGTFREEDSPEMCLLCRTGCPRGMVKVGDCTPWSDIECVHKEEFESKYGPPCPPCPAPEFLGGPSVFLFPPKPKDTLMISRTPEVTCVVVDVSQEDPEVQFNWYVDGVEVHNAKTKPREEQFNSTYRVVSVLTVLHQDWLNGKEYKCKVSNKGLPSSIEKTISKAKGQPREPQVYTLPPSQEEMTKNQVSLTCLVKGFYPSDIAVEWESNGQPENNYKTTPPVLDSDGSFFLYSRLTVDKSRWQEGNVFSCSVMHEALHNHYTQKSLSLSLGK

SEQ ID NO: 67 - protein, 358 aa, synthetic construct
  REGION 1..358: note = YF01M85G4
ITQQDLAPQQRAAPQQKRSSPSEGLCPPGHHISEDGRDCISCKYGQDYSTHWNDLLFCLRCTRCDSGEVELSPCTTTRNTVCQCEEGTFREEDSPEMCSSCRTGCPRGMVKVGDCTPWSDIECVHKEEFESKYGPPCPPCPAPEFLGGPSVFLFPPKPKDTLMISRTPEVTCVVVDVSQEDPEVQFNWYVDGVEVHNAKTKPREEQFNSTYRVVSVLTVLHQDWLNGKEYKCKVSNKGLPSSIEKTISKAKGQPREPQVYTLPPSQEEMTKNQVSLTCLVKGFYPSDIAVEWESNGQPENNYKTTPPVLDSDGSFFLYSRLTVDKSRWQEGNVFSCSVMHEALHNHYTQKSLSLSLGK

SEQ ID NO: 68 - protein, 358 aa, synthetic construct
  REGION 1..358: note = YF01M86G4
ITQQDLAPQQRAAPQQKRSSPSEGLCPPGHHISEDGRDCISCKYGQDYSTHWNDLLFCLRCTRCDSGEVELSPCTTTRNTVCQCEEGTFREEDSPEMCWWCRTGCPRGMVKVGDCTPWSDIECVHKEEFESKYGPPCPPCPAPEFLGGPSVFLFPPKPKDTLMISRTPEVTCVVVDVSQEDPEVQFNWYVDGVEVHNAKTKPREEQFNSTYRVVSVLTVLHQDWLNGKEYKCKVSNKGLPSSIEKTISKAKGQPREPQVYTLPPSQEEMTKNQVSLTCLVKGFYPSDIAVEWESNGQPENNYKTTPPVLDSDGSFFLYSRLTVDKSRWQEGNVFSCSVMHEALHNHYTQKSLSLSLGK

SEQ ID NO: 69 - protein, 358 aa, synthetic construct
  REGION 1..358: note = YF01M87G4
ITQQDLAPQQRAAPQQKRSSPSEGLCPPGHHISEDGRDCISCKYGQDYSTHWNDLLFCLRCTRCDSGEVELSPCTTTRNTVCQCEEGTFREEDSPEMCYYCRTGCPRGMVKVGDCTPWSDIECVHKEEFESKYGPPCPPCPAPEFLGGPSVFLFPPKPKDTLMISRTPEVTCVVVDVSQEDPEVQFNWYVDGVEVHNAKTKPREEQFNSTYRVVSVLTVLHQDWLNGKEYKCKVSNKGLPSSIEKTISKAKGQPREPQVYTLPPSQEEMTKNQVSLTCLVKGFYPSDIAVEWESNGQPENNYKTTPPVLDSDGSFFLYSRLTVDKSRWQEGNVFSCSVMHEALHNHYTQKSLSLSLGK

SEQ ID NO: 70 - protein, 361 aa, synthetic construct
  REGION 1..361: note = YF01M3G1m
ITQQDLAPQQRAAPQQKRSSPSEGLCPPGHHISEDGRDCISCKYGQDYSTHWNDLLFCAACTRCDSGEVELSPCTTTRNTVCQCEEGTFREEDSPEMCRKCRTGCPRGMVKVGDCTPWSDIECVHKEEFEPKSCDKTHTCPPCPAPELLGGPSVFLFPPKPKDTLMISRTPEVTCVVVAVSHEDPEVKFNWYVDGVEVHNAKTKPREEQYNSTYRVVSVLTVLHQDWLNGKEYKCKVSNKALPAPIEKTISKAKGQPREPQVYTLPPSRDELTKNQVSLTCLVKGFYPSDIAVEWESNGQPENNYKTTPPVLDSDGSFFLYSKLTVDKSRWQQGNVFSCSVMHEALHNHYTQKSLSLSPGK

SEQ ID NO: 71 - protein, 361 aa, synthetic construct
  REGION 1..361: note = YF01M5G1m
ITQQDLAPQQRAAPQQKRSSPSEGLCPPGHHISEDGRDCISCKYGQDYSTHWNDLLFCGGCTRCDSGEVELSPCTTTRNTVCQCEEGTFREEDSPEMCRKCRTGCPRGMVKVGDCTPWSDIECVHKEEFEPKSCDKTHTCPPCPAPELLGGPSVFLFPPKPKDTLMISRTPEVTCVVVAVSHEDPEVKFNWYVDGVEVHNAKTKPREEQYNSTYRVVSVLTVLHQDWLNGKEYKCKVSNKALPAPIEKTISKAKGQPREPQVYTLPPSRDELTKNQVSLTCLVKGFYPSDIAVEWESNGQPENNYKTTPPVLDSDGSFFLYSKLTVDKSRWQQGNVFSCSVMHEALHNHYTQKSLSLSPGK

SEQ ID NO: 72 - protein, 361 aa, synthetic construct
  REGION 1..361: note = YF01M14G1m
ITQQDLAPQQRAAPQQKRSSPSEGLCPPGHHISEDGRDCISCKYGQDYSTHWNDLLFCVVCTRCDSGEVELSPCTTTRNTVCQCEEGTFREEDSPEMCRKCRTGCPRGMVKVGDCTPWSDIECVHKEEFEPKSCDKTHTCPPCPAPELLGGPSVFLFPPKPKDTLMISRTPEVTCVVVAVSHEDPEVKFNWYVDGVEVHNAKTKPREEQYNSTYRVVSVLTVLHQDWLNGKEYKCKVSNKALPAPIEKTISKAKGQPREPQVYTLPPSRDELTKNQVSLTCLVKGFYPSDIAVEWESNGQPENNYKTTPPVLDSDGSFFLYSKLTVDKSRWQQGNVFSCSVMHEALHNHYTQKSLSLSPGK

SEQ ID NO: 73 - protein, 361 aa, synthetic construct
  REGION 1..361: note = YF01M16G1m
ITQQDLAPQQRAAPQQKRSSPSEGLCPPGHHISEDGRDCISCKYGQDYSTHWNDLLFCLLCTRCDSGEVELSPCTTTRNTVCQCEEGTFREEDSPEMCRKCRTGCPRGMVKVGDCTPWSDIECVHKEEFEPKSCDKTHTCPPCPAPELLGGPSVFLFPPKPKDTLMISRTPEVTCVVVAVSHEDPEVKFNWYVDGVEVHNAKTKPREEQYNSTYRVVSVLTVLHQDWLNGKEYKCKVSNKALPAPIEKTISKAKGQPREPQVYTLPPSRDELTKNQVSLTCLVKGFYPSDIAVEWESNGQPENNYKTTPPVLDSDGSFFLYSKLTVDKSRWQQGNVFSCSVMHEALHNHYTQKSLSLSPGK

SEQ ID NO: 74 - protein, 361 aa, synthetic construct
  REGION 1..361: note = YF01M29G1m
ITQQDLAPQQRAAPQQKRSSPSEGLCPPGHHISEDGRDCISCKYGQDYSTHWNDLLFCSSCTRCDSGEVELSPCTTTRNTVCQCEEGTFREEDSPEMCRKCRTGCPRGMVKVGDCTPWSDIECVHKEEFEPKSCDKTHTCPPCPAPELLGGPSVFLFPPKPKDTLMISRTPEVTCVVVAVSHEDPEVKFNWYVDGVEVHNAKTKPREEQYNSTYRVVSVLTVLHQDWLNGKEYKCKVSNKALPAPIEKTISKAKGQPREPQVYTLPPSRDELTKNQVSLTCLVKGFYPSDIAVEWESNGQPENNYKTTPPVLDSDGSFFLYSKLTVDKSRWQQGNVFSCSVMHEALHNHYTQKSLSLSPGK

SEQ ID NO: 75 - protein, 361 aa, synthetic construct
  REGION 1..361: note = YF01M36G1m
ITQQDLAPQQRAAPQQKRSSPSEGLCPPGHHISEDGRDCISCKYGQDYSTHWNDLLFCWWCTRCDSGEVELSPCTTTRNTVCQCEEGTFREEDSPEMCRKCRTGCPRGMVKVGDCTPWSDIECVHKEEFEPKSCDKTHTCPPCPAPELLGGPSVFLFPPKPKDTLMISRTPEVTCVVVAVSHEDPEVKFNWYVDGVEVHNAKTKPREEQYNSTYRVVSVLTVLHQDWLNGKEYKCKVSNKALPAPIEKTISKAKGQPREPQVYTLPPSRDELTKNQVSLTCLVKGFYPSDIAVEWESNGQPENNYKTTPPVLDSDGSFFLYSKLTVDKSRWQQGNVFSCSVMHEALHNHYTQKSLSLSPGK

SEQ ID NO: 76 - protein, 361 aa, synthetic construct
  REGION 1..361: note = YF01M42G1m
ITQQDLAPQQRAAPQQKRSSPSEGLCPPGHHISEDGRDCISCKYGQDYSTHWNDLLFCYYCTRCDSGEVELSPCTTTRNTVCQCEEGTFREEDSPEMCRKCRTGCPRGMVKVGDCTPWSDIECVHKEEFEPKSCDKTHTCPPCPAPELLGGPSVFLFPPKPKDTLMISRTPEVTCVVVAVSHEDPEVKFNWYVDGVEVHNAKTKPREEQYNSTYRVVSVLTVLHQDWLNGKEYKCKVSNKALPAPIEKTISKAKGQPREPQVYTLPPSRDELTKNQVSLTCLVKGFYPSDIAVEWESNGQPENNYKTTPPVLDSDGSFFLYSKLTVDKSRWQQGNVFSCSVMHEALHNHYTQKSLSLSPGK

SEQ ID NO: 77 - protein, 361 aa, synthetic construct
  REGION 1..361: note = YF01M47G1m
ITQQDLAPQQRAAPQQKRSSPSEGLCPPGHHISEDGRDCISCKYGQDYSTHWNDLLFCLRCTRCDSGEVELSPCTTTRNTVCQCEEGTFREEDSPEMCAACRTGCPRGMVKVGDCTPWSDIECVHKEEFEPKSCDKTHTCPPCPAPELLGGPSVFLFPPKPKDTLMISRTPEVTCVVVAVSHEDPEVKFNWYVDGVEVHNAKTKPREEQYNSTYRVVSVLTVLHQDWLNGKEYKCKVSNKALPAPIEKTISKAKGQPREPQVYTLPPSRDELTKNQVSLTCLVKGFYPSDIAVEWESNGQPENNYKTTPPVLDSDGSFFLYSKLTVDKSRWQQGNVFSCSVMHEALHNHYTQKSLSLSPGK

SEQ ID NO: 78 - protein, 361 aa, synthetic construct
  REGION 1..361: note = YF01M51G1m
ITQQDLAPQQRAAPQQKRSSPSEGLCPPGHHLSESGRDCISCKYGQDYSNHWNHLLFCLRCTRCDSGEVELSPCTTTRNTVCQCEEGTFREENSPEMCRKCRTGCPRGMVKVGDCTPWSDIECVHKEEFEPKSCDKTHTCPPCPAPELLGGPSVFLFPPKPKDTLMISRTPEVTCVVVAVSHEDPEVKFNWYVDGVEVHNAKTKPREEQYNSTYRVVSVLTVLHQDWLNGKEYKCKVSNKALPAPIEKTISKAKGQPREPQVYTLPPSRDELTKNQVSLTCLVKGFYPSDIAVEWESNGQPENNYKTTPPVLDSDGSFFLYSKLTVDKSRWQQGNVFSCSVMHEALHNHYTQKSLSLSPGK

SEQ ID NO: 79 - protein, 361 aa, synthetic construct
  REGION 1..361: note = YF01M52G1m
ITQQDLAPQQRAAPQQKRSSPSEGLCPPGHHASESGRDCISCKYGQDYSNHWNSLLFCVRCTRCDSGEVELSPCTTTRNTVCQCEEGTFRESDSPEMCRKCRTGCPRGMVKVGDCTPWSDIECVHKEEFEPKSCDKTHTCPPCPAPELLGGPSVFLFPPKPKDTLMISRTPEVTCVVVAVSHEDPEVKFNWYVDGVEVHNAKTKPREEQYNSTYRVVSVLTVLHQDWLNGKEYKCKVSNKALPAPIEKTISKAKGQPREPQVYTLPPSRDELTKNQVSLTCLVKGFYPSDIAVEWESNGQPENNYKTTPPVLDSDGSFFLYSKLTVDKSRWQQGNVFSCSVMHEALHNHYTQKSLSLSPGK

SEQ ID NO: 80 - protein, 361 aa, synthetic construct
  REGION 1..361: note = YF01M54G1m
ITQQDLAPQQRAAPQQKRSSPSEGLCPPGHHASNNGRDCISCKYGQDYSTHWNQLLFCLRCTRCDSGEVELSPCTTTRNTVCQCEEGTFREYDSPEMCRKCRTGCPRGMVKVGDCTPWSDIECVHKEEFEPKSCDKTHTCPPCPAPELLGGPSVFLFPPKPKDTLMISRTPEVTCVVVAVSHEDPEVKFNWYVDGVEVHNAKTKPREEQYNSTYRVVSVLTVLHQDWLNGKEYKCKVSNKALPAPIEKTISKAKGQPREPQVYTLPPSRDELTKNQVSLTCLVKGFYPSDIAVEWESNGQPENNYKTTPPVLDSDGSFFLYSKLTVDKSRWQQGNVFSCSVMHEALHNHYTQKSLSLSPGK

SEQ ID NO: 81 - protein, 361 aa, synthetic construct
  REGION 1..361: note = YF01M62G1m
ITQQDLAPQQRAAPQQKRSSPSEGLCPPGHHASQSGRDCISCKYGQDYSSHWNSLLFCVRCTRCDSGEVELSPCTTTRNTVCQCEEGTFREEKSPEMCRKCRTGCPRGMVKVGDCTPWSDIECVHKEEFEPKSCDKTHTCPPCPAPELLGGPSVFLFPPKPKDTLMISRTPEVTCVVVAVSHEDPEVKFNWYVDGVEVHNAKTKPREEQYNSTYRVVSVLTVLHQDWLNGKEYKCKVSNKALPAPIEKTISKAKGQPREPQVYTLPPSRDELTKNQVSLTCLVKGFYPSDIAVEWESNGQPENNYKTTPPVLDSDGSFFLYSKLTVDKSRWQQGNVFSCSVMHEALHNHYTQKSLSLSPGK

SEQ ID NO: 82 - protein, 361 aa, synthetic construct
  REGION 1..361: note = YF01M63G1m
ITQQDLAPQQRAAPQQKRSSPSEGLCPPGHHISESGRDCISCKYGQDYSNHWNELLFCIRCTRCDSGEVELSPCTTTRNTVCQCEEGTFREEESPEMCYKCRTGCPRGMVKVGDCTPWSDIECVHKEEFEPKSCDKTHTCPPCPAPELLGGPSVFLFPPKPKDTLMISRTPEVTCVVVAVSHEDPEVKFNWYVDGVEVHNAKTKPREEQYNSTYRVVSVLTVLHQDWLNGKEYKCKVSNKALPAPIEKTISKAKGQPREPQVYTLPPSRDELTKNQVSLTCLVKGFYPSDIAVEWESNGQPENNYKTTPPVLDSDGSFFLYSKLTVDKSRWQQGNVFSCSVMHEALHNHYTQKSLSLSPGK

SEQ ID NO: 83 - protein, 361 aa, synthetic construct
  REGION 1..361: note = YF01M64G1m
ITQQDLAPQQRAAPQQKRSSPSEGLCPPGHHISESGRDCISCKYGQDYSTHWNNLLFCLRCTRCDSGEVELSPCTTTRNTVCQCEEGTFREEESPEMCRKCRTGCPRGMVKVGDCTPWSDIECVHKEEFEPKSCDKTHTCPPCPAPELLGGPSVFLFPPKPKDTLMISRTPEVTCVVVAVSHEDPEVKFNWYVDGVEVHNAKTKPREEQYNSTYRVVSVLTVLHQDWLNGKEYKCKVSNKALPAPIEKTISKAKGQPREPQVYTLPPSRDELTKNQVSLTCLVKGFYPSDIAVEWESNGQPENNYKTTPPVLDSDGSFFLYSKLTVDKSRWQQGNVFSCSVMHEALHNHYTQKSLSLSPGK

SEQ ID NO: 84 - protein, 361 aa, synthetic construct
  REGION 1..361: note = YF01M65G1m
ITQQDLAPQQRAAPQQKRSSPSEGLCPPGHHVSENGRDCISCKYGQDYSTHWNDLLFCLRCTRCDSGEVELSPCTTTRNTVCQCEEGTFREEDSPEMCYKCRTGCPRGMVKVGDCTPWSDIECVHKEEFEPKSCDKTHTCPPCPAPELLGGPSVFLFPPKPKDTLMISRTPEVTCVVVAVSHEDPEVKFNWYVDGVEVHNAKTKPREEQYNSTYRVVSVLTVLHQDWLNGKEYKCKVSNKALPAPIEKTISKAKGQPREPQVYTLPPSRDELTKNQVSLTCLVKGFYPSDIAVEWESNGQPENNYKTTPPVLDSDGSFFLYSKLTVDKSRWQQGNVFSCSVMHEALHNHYTQKSLSLSPGK

SEQ ID NO: 85 - protein, 361 aa, synthetic construct
  REGION 1..361: note = YF01M66G1m
ITQQDLAPQQRAAPQQKRSSPSEGLCPPGHHISEDGRDCISCKYGQDYSSHWQDLLYCLRCTRCDSGEVELSPCTTTRNTVCQCEEGTFREEDSPEMCRKCRTGCPRGMVKVGDCTPWSDIECVHKEEFEPKSCDKTHTCPPCPAPELLGGPSVFLFPPKPKDTLMISRTPEVTCVVVAVSHEDPEVKFNWYVDGVEVHNAKTKPREEQYNSTYRVVSVLTVLHQDWLNGKEYKCKVSNKALPAPIEKTISKAKGQPREPQVYTLPPSRDELTKNQVSLTCLVKGFYPSDIAVEWESNGQPENNYKTTPPVLDSDGSFFLYSKLTVDKSRWQQGNVFSCSVMHEALHNHYTQKSLSLSPGK

SEQ ID NO: 86 - protein, 361 aa, synthetic construct
  REGION 1..361: note = YF01M67G1m
ITQQDLAPQQRAAPQQKRSSPSEGLCPPGHHISEDGRDCISCKYGQDYSTHWNDLLFCVRCTRCDSGEVELSPCTTTRNTVCQCEEGTFREQDSPSMCRKCRTGCPRGMVKVGDCTPWSDIECVHKEEFEPKSCDKTHTCPPCPAPELLGGPSVFLFPPKPKDTLMISRTPEVTCVVVAVSHEDPEVKFNWYVDGVEVHNAKTKPREEQYNSTYRVVSVLTVLHQDWLNGKEYKCKVSNKALPAPIEKTISKAKGQPREPQVYTLPPSRDELTKNQVSLTCLVKGFYPSDIAVEWESNGQPENNYKTTPPVLDSDGSFFLYSKLTVDKSRWQQGNVFSCSVMHEALHNHYTQKSLSLSPGK

SEQ ID NO: 87 - protein, 361 aa, synthetic construct
  REGION 1..361: note = YF01M82G1m
ITQQDLAPQQRAAPQQKRSSPSEGLCPPGHHISEDGRDCISCKYGQDYSTHWNDLLFCLRCTRCDSGEVELSPCTTTRNTVCQCEEGTFREEDSPEMCGGCRTGCPRGMVKVGDCTPWSDIECVHKEEFEPKSCDKTHTCPPCPAPELLGGPSVFLFPPKPKDTLMISRTPEVTCVVVAVSHEDPEVKFNWYVDGVEVHNAKTKPREEQYNSTYRVVSVLTVLHQDWLNGKEYKCKVSNKALPAPIEKTISKAKGQPREPQVYTLPPSRDELTKNQVSLTCLVKGFYPSDIAVEWESNGQPENNYKTTPPVLDSDGSFFLYSKLTVDKSRWQQGNVFSCSVMHEALHNHYTQKSLSLSPGK

SEQ ID NO: 88 - protein, 361 aa, synthetic construct
  REGION 1..361: note = YF01M83G1m
ITQQDLAPQQRAAPQQKRSSPSEGLCPPGHHISEDGRDCISCKYGQDYSTHWNDLLFCLRCTRCDSGEVELSPCTTTRNTVCQCEEGTFREEDSPEMCVVCRTGCPRGMVKVGDCTPWSDIECVHKEEFEPKSCDKTHTCPPCPAPELLGGPSVFLFPPKPKDTLMISRTPEVTCVVVAVSHEDPEVKFNWYVDGVEVHNAKTKPREEQYNSTYRVVSVLTVLHQDWLNGKEYKCKVSNKALPAPIEKTISKAKGQPREPQVYTLPPSRDELTKNQVSLTCLVKGFYPSDIAVEWESNGQPENNYKTTPPVLDSDGSFFLYSKLTVDKSRWQQGNVFSCSVMHEALHNHYTQKSLSLSPGK

SEQ ID NO: 89 - protein, 361 aa, synthetic construct
  REGION 1..361: note = YF01M84G1m
ITQQDLAPQQRAAPQQKRSSPSEGLCPPGHHISEDGRDCISCKYGQDYSTHWNDLLFCLRCTRCDSGEVELSPCTTTRNTVCQCEEGTFREEDSPEMCLLCRTGCPRGMVKVGDCTPWSDIECVHKEEFEPKSCDKTHTCPPCPAPELLGGPSVFLFPPKPKDTLMISRTPEVTCVVVAVSHEDPEVKFNWYVDGVEVHNAKTKPREEQYNSTYRVVSVLTVLHQDWLNGKEYKCKVSNKALPAPIEKTISKAKGQPREPQVYTLPPSRDELTKNQVSLTCLVKGFYPSDIAVEWESNGQPENNYKTTPPVLDSDGSFFLYSKLTVDKSRWQQGNVFSCSVMHEALHNHYTQKSLSLSPGK

SEQ ID NO: 90 - protein, 361 aa, synthetic construct
  REGION 1..361: note = YF01M85G1m
ITQQDLAPQQRAAPQQKRSSPSEGLCPPGHHISEDGRDCISCKYGQDYSTHWNDLLFCLRCTRCDSGEVELSPCTTTRNTVCQCEEGTFREEDSPEMCSSCRTGCPRGMVKVGDCTPWSDIECVHKEEFEPKSCDKTHTCPPCPAPELLGGPSVFLFPPKPKDTLMISRTPEVTCVVVAVSHEDPEVKFNWYVDGVEVHNAKTKPREEQYNSTYRVVSVLTVLHQDWLNGKEYKCKVSNKALPAPIEKTISKAKGQPREPQVYTLPPSRDELTKNQVSLTCLVKGFYPSDIAVEWESNGQPENNYKTTPPVLDSDGSFFLYSKLTVDKSRWQQGNVFSCSVMHEALHNHYTQKSLSLSPGK

SEQ ID NO: 91 - protein, 361 aa, synthetic construct
  REGION 1..361: note = YF01M86G1m
ITQQDLAPQQRAAPQQKRSSPSEGLCPPGHHISEDGRDCISCKYGQDYSTHWNDLLFCLRCTRCDSGEVELSPCTTTRNTVCQCEEGTFREEDSPEMCWWCRTGCPRGMVKVGDCTPWSDIECVHKEEFEPKSCDKTHTCPPCPAPELLGGPSVFLFPPKPKDTLMISRTPEVTCVVVAVSHEDPEVKFNWYVDGVEVHNAKTKPREEQYNSTYRVVSVLTVLHQDWLNGKEYKCKVSNKALPAPIEKTISKAKGQPREPQVYTLPPSRDELTKNQVSLTCLVKGFYPSDIAVEWESNGQPENNYKTTPPVLDSDGSFFLYSKLTVDKSRWQQGNVFSCSVMHEALHNHYTQKSLSLSPGK

SEQ ID NO: 92 - protein, 361 aa, synthetic construct
  REGION 1..361: note = YF01M87G1m
ITQQDLAPQQRAAPQQKRSSPSEGLCPPGHHISEDGRDCISCKYGQDYSTHWNDLLFCLRCTRCDSGEVELSPCTTTRNTVCQCEEGTFREEDSPEMCYYCRTGCPRGMVKVGDCTPWSDIECVHKEEFEPKSCDKTHTCPPCPAPELLGGPSVFLFPPKPKDTLMISRTPEVTCVVVAVSHEDPEVKFNWYVDGVEVHNAKTKPREEQYNSTYRVVSVLTVLHQDWLNGKEYKCKVSNKALPAPIEKTISKAKGQPREPQVYTLPPSRDELTKNQVSLTCLVKGFYPSDIAVEWESNGQPENNYKTTPPVLDSDGSFFLYSKLTVDKSRWQQGNVFSCSVMHEALHNHYTQKSLSLSPGK

SEQ ID NO: 93 - protein, 359 aa, synthetic construct
  REGION 1..359: note = YF01 (human DR5 variant 1 truncated domain not including signal peptide)-IgG1
ITQQDLAPQQRAAPQQKRSSPSEGLCPPGHHISEDGRDCISCKYGQDYSTHWNDLLFCLRCTRCDSGEVELSPCTTTRNTVCQCEEGTFREEDSPEMCRKCRTGCPRGMVKVGDCTPWSDIECVHKEEPKSCDKTHTCPPCPAPELLGGPSVFLFPPKPKDTLMISRTPEVTCVVVDVSHEDPEVKFNWYVDGVEVHNAKTKPREEQYNSTYRVVSVLTVLHQDWLNGKEYKCKVSNKALPAPIEKTISKAKGQPREPQVYTLPPSRDELTKNQVSLTCLVKGFYPSDIAVEWESNGQPENNYKTTPPVLDSDGSFFLYSKLTVDKSRWQQGNVFSCSVMHEALHNHYTQKSLSLSPGK

SEQ ID NO: 94 - protein, 127 aa, synthetic construct
  REGION 1..127: note = human DR5 variant 1 truncated domain not including signal peptide
ITQQDLAPQQRAAPQQKRSSPSEGLCPPGHHISEDGRDCISCKYGQDYSTHWNDLLFCLRCTRCDSGEVELSPCTTTRNTVCQCEEGTFREEDSPEMCRKCRTGCPRGMVKVGDCTPWSDIECVHKE

SEQ ID NO: 95 - protein, 440 aa, synthetic construct
  REGION 1..440: note = human DR5 variant 1
MEQRGQNAPAASGARKRHGPGPREARGARPGPRVPKTLVLVVAAVLLLVSAESALITQQDLAPQQRAAPQQKRSSPSEGLCPPGHHISEDGRDCISCKYGQDYSTHWNDLLFCLRCTRCDSGEVELSPCTTTRNTVCQCEEGTFREEDSPEMCRKCRTGCPRGMVKVGDCTPWSDIECVHKESGTKHSGEVPAVEETVTSSPGTPASPCSLSGIIIGVTVAAVVLIVAVFVCKSLLWKKVLPYLKGICSGGGGDPERVDRSSQRPGAEDNVLNEIVSILQPTQVPEQEMEVQEPAEPTGVNMLSPGESEHLLEPAEAERSQRRRLLVPANEGDPTETLRQCFDDFADLVPFDSWEPLMRKLGLMDNEIKVAKAEAAGHRDTLYTMLIKWVNKTGRDASVHTLLDALETLGERLAKQKIEDHLLSSGKFMYLEGNADSAMS

SEQ ID NO: 96 - protein, 182 aa, synthetic construct
  REGION 1..182: note = human DR5 variant 1 extracellular domain including signal peptide
MEQRGQNAPAASGARKRHGPGPREARGARPGPRVPKTLVLVVAAVLLLVSAESALITQQDLAPQQRAAPQQKRSSPSEGLCPPGHHISEDGRDCISCKYGQDYSTHWNDLLFCLRCTRCDSGEVELSPCTTTRNTVCQCEEGTFREEDSPEMCRKCRTGCPRGMVKVGDCTPWSDIECVHKE

SEQ ID NO: 97 - protein, 232 aa, synthetic construct
  REGION 1..232: note = Human IgG1-Fc
EPKSCDKTHTCPPCPAPELLGGPSVFLFPPKPKDTLMISRTPEVTCVVVDVSHEDPEVKFNWYVDGVEVHNAKTKPREEQYNSTYRVVSVLTVLHQDWLNGKEYKCKVSNKALPAPIEKTISKAKGQPREPQVYTLPPSRDELTKNQVSLTCLVKGFYPSDIAVEWESNGQPENNYKTTPPVLDSDGSFFLYSKLTVDKSRWQQGNVFSCSVMHEALHNHYTQKSLSLSPGK

SEQ ID NO: 98 - protein, 229 aa, synthetic construct
  REGION 1..229: note = Human IgG4-Fc
ESKYGPPCPPCPAPEFLGGPSVFLFPPKPKDTLMISRTPEVTCVVVDVSQEDPEVQFNWYVDGVEVHNAKTKPREEQFNSTYRVVSVLTVLHQDWLNGKEYKCKVSNKGLPSSIEKTISKAKGQPREPQVYTLPPSQEEMTKNQVSLTCLVKGFYPSDIAVEWESNGQPENNYKTTPPVLDSDGSFFLYSRLTVDKSRWQEGNVFSCSVMHEALHNHYTQKSLSLSLGK

SEQ ID NO: 99 - protein, 232 aa, synthetic construct
  REGION 1..232: note = Human IgG1-Fc mutant D265A
EPKSCDKTHTCPPCPAPELLGGPSVFLFPPKPKDTLMISRTPEVTCVVVAVSHEDPEVKFNWYVDGVEVHNAKTKPREEQYNSTYRVVSVLTVLHQDWLNGKEYKCKVSNKALPAPIEKTISKAKGQPREPQVYTLPPSRDELTKNQVSLTCLVKGFYPSDIAVEWESNGQPENNYKTTPPVLDSDGSFFLYSKLTVDKSRWQQGNVFSCSVMHEALHNHYTQKSLSLSPGK